European Patent Application EP 4 497 829 A1, published January 29, 2025. Title: Minimal precursors of syn-tasiRNAs. Applicant: CONSEJO SUPERIOR DE INVESTIGACIONES CIENTIFICAS (CSIC). Application EP. The sequence listing filed with the application follows.

SEQUENCE LISTING (79 sequences)

SEQ ID NO: 1 - RNA, 11 nt, Arabidopsis thaliana
  source 1..11: mol_type = other RNA
tagaccattta

SEQ ID NO: 2 - RNA, 22 nt, synthetic construct
  source 1..22: mol_type = other RNA
gtgatttttctctacaagcgaa

SEQ ID NO: 3 - RNA, 22 nt, synthetic construct
  source 1..22: mol_type = other RNA
gtggtatggggggagtcgggaa

SEQ ID NO: 4 - RNA, 22 nt, synthetic construct
  source 1..22: mol_type = other RNA
aaacatttacaagtcacctgta

SEQ ID NO: 5 - RNA, 22 nt, synthetic construct
  source 1..22: mol_type = other RNA
ggcatgggcggtgtaggcaaga

SEQ ID NO: 6 - RNA, 22 nt, synthetic construct
  source 1..22: mol_type = other RNA
aaagatactcggaaaacattta

SEQ ID NO: 7 - RNA, 22 nt, Arabidopsis thaliana
  source 1..22: mol_type = other RNA
ttcgcttgcagagagaaatcac

SEQ ID NO: 8 - RNA, 22 nt, Arabidopsis thaliana
  source 1..22: mol_type = other RNA
ttcccgactccccccataccac

SEQ ID NO: 9 - RNA, 22 nt, Nicotiana benthamiana
  source 1..22: mol_type = other RNA
tacaggtgacttgtaaatgttt

SEQ ID NO: 10 - RNA, 22 nt, Solanum lycopersicum
  source 1..22: mol_type = other RNA
tcttgcctacaccgcccatgcc

SEQ ID NO: 11 - RNA, 21 nt, synthetic construct
  source 1..21: mol_type = other RNA
tgtaagacgtgattgtgtcct

SEQ ID NO: 12 - RNA, 21 nt, synthetic construct
  source 1..21: mol_type = other RNA
tatcagctctgggtgaatcgg

SEQ ID NO: 13 - RNA, 21 nt, synthetic construct
  source 1..21: mol_type = other RNA
ttggtatagtggggcataccg

SEQ ID NO: 14 - RNA, 21 nt, synthetic construct
  source 1..21: mol_type = other RNA
tcagagtgcacaatccatctt

SEQ ID NO: 15 - RNA, 21 nt, synthetic construct
  source 1..21: mol_type = other RNA
tcggccgctgggcactcccct

SEQ ID NO: 16 - RNA, 21 nt, synthetic construct
  source 1..21: mol_type = other RNA
tgcgggcgcgaggaaggacag

SEQ ID NO: 17 - RNA, 21 nt, synthetic construct
  source 1..21: mol_type = other RNA
tttccaccgggtagtagccgt

SEQ ID NO: 18 - RNA, 21 nt, synthetic construct
  source 1..21: mol_type = other RNA
ttagttccgaggaaccaactc

SEQ ID NO: 19 - RNA, 21 nt, synthetic construct
  source 1..21: mol_type = other RNA
tcaagggctaaacaccctcgg

SEQ ID NO: 20 - RNA, 21 nt, synthetic construct
  source 1..21: mol_type = other RNA
tggaaccgcagttggttcctg

SEQ ID NO: 21 - RNA, 21 nt, synthetic construct
  source 1..21: mol_type = other RNA
tgaagctcccgagaaccgcta

SEQ ID NO: 22 - RNA, 21 nt, synthetic construct
  source 1..21: mol_type = other RNA
tgtcgcttcggctactacccc

SEQ ID NO: 23 - RNA, 21 nt, synthetic construct
  source 1..21: mol_type = other RNA
tgtccttcctcgcgcccgcac

SEQ ID NO: 24 - RNA, 21 nt, synthetic construct
  source 1..21: mol_type = other RNA
tggttcacacctgacctcctc

SEQ ID NO: 25 - RNA, 21 nt, synthetic construct
  source 1..21: mol_type = other RNA
tcccggggaaacctggagcgt

SEQ ID NO: 26 - RNA, 21 nt, Arabidopsis thaliana
  source 1..21: mol_type = other RNA
gaactagaaaagacattggac

SEQ ID NO: 27 - RNA, 50 nt, Arabidopsis thaliana
  source 1..50: mol_type = other RNA
gatttcgttgggttacggatgttttcgagatgaaacagcattgttttgtt

SEQ ID NO: 28 - RNA, 50 nt, Arabidopsis thaliana
  source 1..50: mol_type = other RNA
atattccaggatatgcaaaagaaaacaatgaatattgttttgaatgtgtt

SEQ ID NO: 29 - RNA, 366 nt, Arabidopsis thaliana
  source 1..366: mol_type = other RNA
aaacctaaacctaaacggctaagcccgacgtcaaataccaaaaagagaaaaacaagagcgccgtcaagctctgcaaatacgatctgtaagtccatcttaacacaaaagtgagatgggttcttagatcatgttccgccgttagatcgagtcatggtcttgtctcatagaaaggtactttcgtttacttcttttgagtatcgagtagagcgtcgtctatagttagtttgagattgcgtttgtcagaagttaggttcaatgtcccggtccaattttcaccagccatgtgtcagtttcgttccttcccgtcctcttctttgatttcgttgggttacggatgttttcgagatgaaacagcattgttttgtt

SEQ ID NO: 30 - RNA, 507 nt, Arabidopsis thaliana
  source 1..507: mol_type = other RNA
atattccaggatatgcaaaagaaaacaatgaatattgttttgaatgtgttcaagtaaatgagattttcaagtcgtctaaagaacagttgctaatacagttacttatttcaataaataattggttctaataatacaaaacatattcgaggatatgcagaaaaaaagatgtttgttattttgaaaagcttgagtagtttctctccgaggtgtagcgaagaagcatcatctactttgtaatgtaattttctttatgttttcactttgtaattttatttgtgttaatgtaccatggccgatatcggttttattgaaagaaaatttatgttacttctgttttggctttgcaatcagttatgctagttttcttataccctttcgtaagcttcctaaggaatcgttcattgatttccactgcttcattgtatattaaaactttacaactgtatcgaccatcatataattctgggtcaagagatgaaaatagaacaccacatcgtaaagtgaaat

SEQ ID NO: 31 - RNA, 22 nt, Solanum lycopersicum
  source 1..22: mol_type = other RNA
taaatgttttccgagtatcttt

SEQ ID NO: 32 - DNA, 21 bp, synthetic construct
  source 1..21: mol_type = other DNA
aggggccatgctaatcttctc

SEQ ID NO: 33 - DNA, 21 bp, synthetic construct
  source 1..21: mol_type = other DNA
ggcctcttcctttataaccaa

SEQ ID NO: 34 - DNA, 21 bp, synthetic construct
  source 1..21: mol_type = other DNA
agggatttccgtgacacttaa

SEQ ID NO: 35 - DNA, 21 bp, synthetic construct
  source 1..21: mol_type = other DNA
aaaaatggctgaggctgatga

SEQ ID NO: 36 - DNA, 19 bp, synthetic construct
  source 1..19: mol_type = other DNA
gaaaaacagccctgggagc

SEQ ID NO: 37 - DNA, 21 bp, synthetic construct
  source 1..21: mol_type = other DNA
catgcacaagtagggacggtt

SEQ ID NO: 38 - DNA, 21 bp, synthetic construct
  source 1..21: mol_type = other DNA
gtcacggaaatcctttgggtt

SEQ ID NO: 39 - DNA, 20 bp, synthetic construct
  source 1..20: mol_type = other DNA
tggaacaacctttggcaatg

SEQ ID NO: 40 - DNA, 20 bp, synthetic construct
  source 1..20: mol_type = other DNA
cgacacgatgaattcctgca

SEQ ID NO: 41 - DNA, 22 bp, synthetic construct
  source 1..22: mol_type = other DNA
gaccctgatgttgatgttcgct

SEQ ID NO: 42 - DNA, 22 bp, synthetic construct
  source 1..22: mol_type = other DNA
gagggatttgaagagagatttc

SEQ ID NO: 43 - DNA, 22 bp, synthetic construct
  source 1..22: mol_type = other DNA
gaccctgatgttgatgttcgct

SEQ ID NO: 44 - DNA, 22 bp, synthetic construct
  source 1..22: mol_type = other DNA
gagggatttgaagagagatttc

SEQ ID NO: 45 - DNA, 21 bp, synthetic construct
  source 1..21: mol_type = other DNA
  modified_base 2: mod_base = OTHER; note = Locked nucleic acid cytosine (LNA-C)
  modified_base 5: mod_base = OTHER; note = Locked nucleic acid guanosine (LNA-G)
  modified_base 8: mod_base = OTHER; note = locked nucleic acid guanosine (LNA-G)
  modified_base 11: mod_base = OTHER; note = locked nucleic acid cytosine (LNA-C)
  modified_base 14: mod_base = OTHER; note = locked nucleic acid cytosine (LNA-C)
  modified_base 17: mod_base = OTHER; note = locked nucleic acid guanosine (LNA-G)
  modified_base 20: mod_base = OTHER; note = locked nucleic acid thymidine (LNA-T)
gcgggaagtccaccacggtta

SEQ ID NO: 46 - DNA, 36 bp, synthetic construct
  source 1..36: mol_type = other DNA
ccccataccacaacaaaacaatgctgtttcatctcg

SEQ ID NO: 47 - DNA, 38 bp, synthetic construct
  source 1..38: mol_type = other DNA
cacttacccgagttaacgccaaacctaaacctaaacgg

SEQ ID NO: 48 - DNA, 39 bp, synthetic construct
  source 1..39: mol_type = other DNA
gtttaatgtcttcgggacatatttcactttacgatgtgg

SEQ ID NO: 49 - DNA, 38 bp, synthetic construct
  source 1..38: mol_type = other DNA
cacttacccgagttaacgccagtagagaagaatctgta

SEQ ID NO: 50 - DNA, 35 bp, synthetic construct
  source 1..35: mol_type = other DNA
gtttaatgtcttcgggacatagtaagaagagccaa

SEQ ID NO: 51 - DNA, 36 bp, synthetic construct
  source 1..36: mol_type = other DNA
ggagtcgggaatagaccatttatgtatgactcccgg

SEQ ID NO: 52 - DNA, 58 bp, synthetic construct
  source 1..58: mol_type = other DNA
caccgtggtatggggggagtcgggaatagaccatttatgtatgactcccggaattcca

SEQ ID NO: 53 - DNA, 58 bp, synthetic construct
  source 1..58: mol_type = other DNA
tggaattccgggagtcatacataaatggtctattcccgactccccccataccacggtg

SEQ ID NO: 54 - DNA, 94 bp, synthetic construct
  source 1..94: mol_type = other DNA
agaggtcagcaccagctagcgtggtatggggggagtcgggaatagaccatttatgtatgactcccggaattccaagggtttgttaagtttccct

SEQ ID NO: 55 - DNA, 94 bp, synthetic construct
  source 1..94: mol_type = other DNA
cacttacccgagttaacgccgtggtatggggggagtcgggaatagaccatttatgtatgactcccggaattccaatgtcccgaagacattaaac

SEQ ID NO: 56 - DNA, 58 bp, synthetic construct
  source 1..58: mol_type = other DNA
caccgtgatttttctctacaagcgaatagaccatttatgcgcttgctgagtttccccc

SEQ ID NO: 57 - DNA, 58 bp, synthetic construct
  source 1..58: mol_type = other DNA
gggggaaactcagcaagcgcataaatggtctattcgcttgtagagaaaaatcacggtg

SEQ ID NO: 58 - DNA, 58 bp, synthetic construct
  source 1..58: mol_type = other DNA
caccgtgatttttctctacaagcgaatagaccatttattaagtgtcacggaaatccct

SEQ ID NO: 59 - DNA, 58 bp, synthetic construct
  source 1..58: mol_type = other DNA
agggatttccgtgacacttaataaatggtctattcgcttgtagagaaaaatcacggtg

SEQ ID NO: 60 - DNA, 58 bp, synthetic construct
  source 1..58: mol_type = other DNA
caccgtgatttttctctacaagcgaatagaccatttattggttataaaggaagaggcc

SEQ ID NO: 61 - DNA, 58 bp, synthetic construct
  source 1..58: mol_type = other DNA
ggcctcttcctttataaccaataaatggtctattcgcttgtagagaaaaatcacggtg

SEQ ID NO: 62 - DNA, 79 bp, synthetic construct
  source 1..79: mol_type = other DNA
caccgtgatttttctctacaagcgaatagaccatttattggttataaaggaagaggcctcccattcgatactgctcgcc

SEQ ID NO: 63 - DNA, 79 bp, synthetic construct
  source 1..79: mol_type = other DNA
ggcgagcagtatcgaatgggaggcctcttcctttataaccaataaatggtctattcgcttgtagagaaaaatcacggtg

SEQ ID NO: 64 - DNA, 79 bp, synthetic construct
  source 1..79: mol_type = other DNA
caccgtgatttttctctacaagcgaatagaccatttatcccattcgatactgctcgccttggttataaaggaagaggcc

SEQ ID NO: 65 - DNA, 79 bp, synthetic construct
  source 1..79: mol_type = other DNA
ggcctcttcctttataaccaaggcgagcagtatcgaatgggataaatggtctattcgcttgtagagaaaaatcacggtg

SEQ ID NO: 66 - DNA, 115 bp, synthetic construct
  source 1..115: mol_type = other DNA
agaggtcagcaccagctagcggcatgggcggtgtaggcaagatagaccatttatcccccttgtatgattcccgctctcaatgtcgattgtcccagagggtttgttaagtttccct

SEQ ID NO: 67 - DNA, 58 bp, synthetic construct
  source 1..58: mol_type = other DNA
tgtaggcatgggcggtgtaggcaagatagaccatttatattgacccacactttgccga

SEQ ID NO: 68 - DNA, 58 bp, synthetic construct
  source 1..58: mol_type = other DNA
aatgtcggcaaagtgtgggtcaatataaatggtctatcttgcctacaccgcccatgcc

SEQ ID NO: 69 - DNA, 58 bp, synthetic construct
  source 1..58: mol_type = other DNA
tgtaggcatgggcggtgtaggcaagatagaccatttatgtatgactcccggaattcca

SEQ ID NO: 70 - DNA, 58 bp, synthetic construct
  source 1..58: mol_type = other DNA
aatgtggaattccgggagtcatacataaatggtctatcttgcctacaccgcccatgcc

SEQ ID NO: 71 - DNA, 22 bp, synthetic construct
  source 1..22: mol_type = other DNA
gggaatcaatcacagtgttggc

SEQ ID NO: 72 - DNA, 22 bp, synthetic construct
  source 1..22: mol_type = other DNA
gctactatggcacgggctgtac

SEQ ID NO: 73 - DNA, 20 bp, synthetic construct
  source 1..20: mol_type = other DNA
tcggtttgctgacctactgg

SEQ ID NO: 74 - DNA, 21 bp, synthetic construct
  source 1..21: mol_type = other DNA
aacctaaaacttcagacacgg

SEQ ID NO: 75 - DNA, 94 bp, synthetic construct
  source 1..94: mol_type = other DNA
agaggtcagcaccagctagcnnnnnnnnnnnnnnnnnnnnnntagaccatttannnnnnnnnnnnnnnnnnnnnagggtttgttaagtttccct

SEQ ID NO: 76 - DNA, 94 bp, synthetic construct
  source 1..94: mol_type = other DNA
cacttacccgagttaacgccnnnnnnnnnnnnnnnnnnnnnntagaccatttannnnnnnnnnnnnnnnnnnnnatgtcccgaagacattaaac

SEQ ID NO: 77 - RNA, 33 nt, synthetic construct
  source 1..33: mol_type = other RNA
gtgatttttctctacaagcgaatagaccattta

SEQ ID NO: 78 - RNA, 33 nt, synthetic construct
  source 1..33: mol_type = other RNA
gtggtatggggggagtcgggaatagaccattta

SEQ ID NO: 79 - RNA, 33 nt, synthetic construct
  source 1..33: mol_type = other RNA
ggcatgggcggtgtaggcaagatagaccattta